European Patent Specification EP 3 609 914 B1, published February 18, 2026. Title: CHIMERIC ANTIGEN RECEPTOR T CELLS TARGETING THE TUMOR MICROENVIRONMENT. Applicant: The General Hospital Corporation. The sequence listing filed with the application follows.

SEQUENCE LISTING (68 sequences)

SEQ ID NO: 1 - protein, 351 aa, Artificial Sequence
  Synthetic Construct
MALPVTALLLPLALLLHAARPDIQMTQSPSSLSASLGDRVTITCQASQSISSYLAWYQQKPGQAPNILIYGASRLKTGVPSRFSGSGSGTSFTLTISGLEAEDAGTYYCQQYASVPVTFGQGTKVELKTTTPAPRPPTPAPTIASQPLSLRPEACRPAAGGAVHTRGLDFACDIYIWAPLAGTCGVLLLSLVITLYCKRGRKKLLYIFKQPFMRPVQTTQEEDGCSCRFPEEEEGGCELRVKFSRSADAPAYQQGQNQLYNELNLGRREEYDVLDKRRGRDPEMGGKPRRKNPQEGLYNELQKDKMAEAYSEIGMKGERRRGKGHDGLYQGLSTATKDTYDALHMQALPPR

SEQ ID NO: 2 - protein, 21 aa, Artificial Sequence
  Synthetic Construct
MALPVTALLLPLALLLHAARP

SEQ ID NO: 3 - protein, 107 aa, Artificial Sequence
  Synthetic Construct
DIQMTQSPSSLSASLGDRVTITCQASQSISSYLAWYQQKPGQAPNILIYGASRLKTGVPSRFSGSGSGTSFTLTISGLEAEDAGTYYCQQYASVPVTFGQGTKVELK

SEQ ID NO: 4 - protein, 69 aa, Artificial Sequence
  Synthetic Construct
TTTPAPRPPTPAPTIASQPLSLRPEACRPAAGGAVHTRGLDFACDIYIWAPLAGTCGVLLLSLVITLYC

SEQ ID NO: 5 - protein, 42 aa, Artificial Sequence
  Synthetic Construct
KRGRKKLLYIFKQPFMRPVQTTQEEDGCSCRFPEEEEGGCEL

SEQ ID NO: 6 - protein, 112 aa, Artificial Sequence
  Synthetic Construct
RVKFSRSADAPAYQQGQNQLYNELNLGRREEYDVLDKRRGRDPEMGGKPRRKNPQEGLYNELQKDKMAEAYSEIGMKGERRRGKGHDGLYQGLSTATKDTYDALHMQALPPR

SEQ ID NO: 7 - protein, 530 aa, Artificial Sequence
  Synthetic Construct
MALPVTALLLPLALLLHAARPMKLWLNWIFLVTLLNDIQCEVKLVESGGGLVQPGGSLSLSCAASGFTFTDYYMSWVRQPPGKALEWLGFIRNKPNGYTTEYSASVKGRFTISRDNSQSILYLQMNVLRAEDSATYYCARYTGGGYFDYWGQGTTLTVSSGGGGSGGGGSGGGGSGGGGSMMSSAQFLGLLLLCFQGTRCDIQMTQTTSSLSASLGDRLTISCRASQDISNYLNWYQQKPDGTVKLLIYYTSRLHSGVPSRFSGSGSGTDYSLTISNLEQADIATYFCQQGDTLPWTFGGGTKLEIKTTTPAPRPPTPAPTIASQPLSLRPEACRPAAGGAVHTRGLDFACDIYIWAPLAGTCGVLLLSLVITLYCKRGRKKLLYIFKQPFMRPVQTTQEEDGCSCRFPEEEEGGCELRVKFSRSADAPAYQQGQNQLYNELNLGRREEYDVLDKRRGRDPEMGGKPRRKNPQEGLYNELQKDKMAEAYSEIGMKGERRRGKGHDGLYQGLSTATKDTYDALHMQALPPR

SEQ ID NO: 8 - protein, 21 aa, Artificial Sequence
  Synthetic Construct
MALPVTALLLPLALLLHAARP

SEQ ID NO: 9 - protein, 286 aa, Artificial Sequence
  Synthetic Construct
MKLWLNWIFLVTLLNDIQCEVKLVESGGGLVQPGGSLSLSCAASGFTFTDYYMSWVRQPPGKALEWLGFIRNKPNGYTTEYSASVKGRFTISRDNSQSILYLQMNVLRAEDSATYYCARYTGGGYFDYWGQGTTLTVSSGGGGSGGGGSGGGGSGGGGSMMSSAQFLGLLLLCFQGTRCDIQMTQTTSSLSASLGDRLTISCRASQDISNYLNWYQQKPDGTVKLLIYYTSRLHSGVPSRFSGSGSGTDYSLTISNLEQADIATYFCQQGDTLPWTFGGGTKLEIK

SEQ ID NO: 10 - protein, 69 aa, Artificial Sequence; identical to SEQ ID NO: 4
  Synthetic Construct

SEQ ID NO: 11 - protein, 42 aa, Artificial Sequence; identical to SEQ ID NO: 5
  Synthetic Construct

SEQ ID NO: 12 - protein, 112 aa, Artificial Sequence; identical to SEQ ID NO: 6
  Synthetic Construct

SEQ ID NO: 13 - protein, 530 aa, Artificial Sequence
  Synthetic Construct
MALPVTALLLPLALLLHAARPMMSSAQFLGLLLLCFQGTRCDIQMTQTTSSLSASLGDRLTISCRASQDISNYLNWYQQKPDGTVKLLIYYTSRLHSGVPSRFSGSGSGTDYSLTISNLEQADIATYFCQQGDTLPWTFGGGTKLEIKGGGGSGGGGSGGGGSGGGGSMKLWLNWIFLVTLLNDIQCEVKLVESGGGLVQPGGSLSLSCAASGFTFTDYYMSWVRQPPGKALEWLGFIRNKPNGYTTEYSASVKGRFTISRDNSQSILYLQMNVLRAEDSATYYCARYTGGGYFDYWGQGTTLTVSSTTTPAPRPPTPAPTIASQPLSLRPEACRPAAGGAVHTRGLDFACDIYIWAPLAGTCGVLLLSLVITLYCKRGRKKLLYIFKQPFMRPVQTTQEEDGCSCRFPEEEEGGCELRVKFSRSADAPAYQQGQNQLYNELNLGRREEYDVLDKRRGRDPEMGGKPRRKNPQEGLYNELQKDKMAEAYSEIGMKGERRRGKGHDGLYQGLSTATKDTYDALHMQALPPR

SEQ ID NO: 14 - protein, 21 aa, Artificial Sequence
  Synthetic Construct
MALPVTALLLPLALLLHAARP

SEQ ID NO: 15 - protein, 286 aa, Artificial Sequence
  Synthetic Construct
MMSSAQFLGLLLLCFQGTRCDIQMTQTTSSLSASLGDRLTISCRASQDISNYLNWYQQKPDGTVKLLIYYTSRLHSGVPSRFSGSGSGTDYSLTISNLEQADIATYFCQQGDTLPWTFGGGTKLEIKGGGGSGGGGSGGGGSGGGGSMKLWLNWIFLVTLLNDIQCEVKLVESGGGLVQPGGSLSLSCAASGFTFTDYYMSWVRQPPGKALEWLGFIRNKPNGYTTEYSASVKGRFTISRDNSQSILYLQMNVLRAEDSATYYCARYTGGGYFDYWGQGTTLTVSS

SEQ ID NO: 16 - protein, 69 aa, Artificial Sequence; identical to SEQ ID NO: 4
  Synthetic Construct

SEQ ID NO: 17 - protein, 42 aa, Artificial Sequence; identical to SEQ ID NO: 5
  Synthetic Construct

SEQ ID NO: 18 - protein, 112 aa, Artificial Sequence; identical to SEQ ID NO: 6
  Synthetic Construct

SEQ ID NO: 19 - protein, 654 aa, Artificial Sequence
  Synthetic Construct
MALPVTALLLPLALLLHAARPQVQLKQSGPGLVQPSQSLSITCTVSGFSLTNYGVHWVRQSPGKGLEWLGVIWSGGNTDYNTPFTSRLSINKDNSKSQVFFKMNSLQSNDTAIYYCARALTYYDYEFAYWGQGTLVTVSAGGGGSGGGGSGGGGSGGGGSDILLTQSPVILSVSPGERVSFSCRASQSIGTNIHWYQQRTNGSPRLLIKYASESISGIPSRFSGSGSGTDFTLSINSVESEDIADYYCQQNNNWPTTFGAGTKLELKTTTPAPRPPTPAPTIASQPLSLRPEACRPAAGGAVHTRGLDFACDIYIWAPLAGTCGVLLLSLVITLYCKRGRKKLLYIFKQPFMRPVQTTQEEDGCSCRFPEEEEGGCELRVKFSRSADAPAYQQGQNQLYNELNLGRREEYDVLDKRRGRDPEMGGKPRRKNPQEGLYNELQKDKMAEAYSEIGMKGERRRGKGHDGLYQGLSTATKDTYDALHMQALPPRPGSGSGATNFSLLKQAGDVEENPGPRTAMETDTLLLWVLLLWVPGSTGDDIQMTQSPSSLSASLGDRVTITCQASQSISSYLAWYQQKPGQAPNILIYGASRLKTGVPSRFSGSGSGTSFTLTISGLEAEDAGTYYCQQYASVPVTFGQGTKVELKHHHHHHSG

SEQ ID NO: 20 - protein, 21 aa, Artificial Sequence
  Synthetic Construct
MALPVTALLLPLALLLHAARP

SEQ ID NO: 21 - protein, 246 aa, Artificial Sequence
  Synthetic Construct
QVQLKQSGPGLVQPSQSLSITCTVSGFSLTNYGVHWVRQSPGKGLEWLGVIWSGGNTDYNTPFTSRLSINKDNSKSQVFFKMNSLQSNDTAIYYCARALTYYDYEFAYWGQGTLVTVSAGGGGSGGGGSGGGGSGGGGSDILLTQSPVILSVSPGERVSFSCRASQSIGTNIHWYQQRTNGSPRLLIKYASESISGIPSRFSGSGSGTDFTLSINSVESEDIADYYCQQNNNWPTTFGAGTKLELK

SEQ ID NO: 22 - protein, 69 aa, Artificial Sequence; identical to SEQ ID NO: 4
  Synthetic Construct

SEQ ID NO: 23 - protein, 42 aa, Artificial Sequence; identical to SEQ ID NO: 5
  Synthetic Construct

SEQ ID NO: 24 - protein, 112 aa, Artificial Sequence; identical to SEQ ID NO: 6
  Synthetic Construct

SEQ ID NO: 25 - protein, 107 aa, Artificial Sequence; identical to SEQ ID NO: 3
  Synthetic Construct

SEQ ID NO: 26 - protein, 1006 aa, Artificial Sequence
  Synthetic Construct
EIQLQQSGAELVKPGASVKLSCTGSGFNIEDYYIHWVKQRTEQGLEWIGRIDPENDETKYGPIFQGRATITADTSSNTVYLQLSSLTSEDTAVYYCAFRGGVYWGPGTTLTVSSGGGGSGGGGSGGGGSHMDVVMTQSPLTLSVAIGQSASISCKSSQSLLDSDGKTYLNWLLQRPGQSPKRLISLVSKLDSGVPDRFTGSGSGTDFTLRISRVEAEDLGIYYCWQGTHFPGTFGGGTKLEIKTTTPAPRPPTPAPTIASQPLSLRPEACRPAAGGAVHTRGLDFACDIYIWAPLAGTCGVLLLSLVITLYCKRGRKKLLYIFKQPFMRPVQTTQEEDGCSCRFPEEEEGGCELRVKFSRSADAPAYQQGQNQLYNELNLGRREEYDVLDKRRGRDPEMGGKPRRKNPQEGLYNELQKDKMAEAYSEIGMKGERRRGKGHDGLYQGLSTATKDTYDALHMQALPPRGSGATNFSLLKQAGDVEENPGPPRMETDTLLLWVLLLWVPGSTGDDILLTQSPVILSVSPGERVSFSCRASQSIGTNIHWYQQRTNGSPRLLIKYASESISGIPSRFSGSGSGTDFTLSINSVESEDIADYYCQQNNNWPTTFGAGTKLELKGGGGSGGGGSGGGGSQVQLKQSGPGLVQPSQSLSITCTVSGFSLTNYGVHWVRQSPGKGLEWLGVIWSGGNTDYNTPFTSRLSINKDNSKSQVFFKMNSLQSNDTAIYYCARALTYYDYEFAYWGQGTLVTVSAGGGGSDIKLQQSGAELARPGASVKMSCKTSGYTFTRYTMHWVKQRPGQGLEWIGYINPSRGYTNYNQKFKDKATLTTDKSSSTAYMQLSSLTSEDSAVYYCARYYDDHYCLDYWGQGTTLTVSSVEGGSGGSGGSGGSGGVDDIQLTQSPAIMSASPGEKVTMTCRASSSVSYMNWYQQKSGTSPKRWIYDTSKVASGVPYRFSGSGSGTSYSLTISSMEAEDAATYYCQQWSSNPLTFGAGTKLELKHHHHHH

SEQ ID NO: 27 - protein, 243 aa, Artificial Sequence
  Synthetic Construct
EIQLQQSGAELVKPGASVKLSCTGSGFNIEDYYIHWVKQRTEQGLEWIGRIDPENDETKYGPIFQGRATITADTSSNTVYLQLSSLTSEDTAVYYCAFRGGVYWGPGTTLTVSSGGGGSGGGGSGGGGSHMDVVMTQSPLTLSVAIGQSASISCKSSQSLLDSDGKTYLNWLLQRPGQSPKRLISLVSKLDSGVPDRFTGSGSGTDFTLRISRVEAEDLGIYYCWQGTHFPGTFGGGTKLEIK

SEQ ID NO: 28 - protein, 69 aa, Artificial Sequence; identical to SEQ ID NO: 4
  Synthetic Construct

SEQ ID NO: 29 - protein, 42 aa, Artificial Sequence; identical to SEQ ID NO: 5
  Synthetic Construct

SEQ ID NO: 30 - protein, 112 aa, Artificial Sequence; identical to SEQ ID NO: 6
  Synthetic Construct

SEQ ID NO: 31 - protein, 22 aa, Artificial Sequence
  Synthetic Construct
GSGATNFSLLKQAGDVEENPGP

SEQ ID NO: 32 - protein, 21 aa, Artificial Sequence
  Synthetic Construct
METDTLLLWVLLLWVPGSTGD

SEQ ID NO: 33 - protein, 241 aa, Artificial Sequence
  Synthetic Construct
DILLTQSPVILSVSPGERVSFSCRASQSIGTNIHWYQQRTNGSPRLLIKYASESISGIPSRFSGSGSGTDFTLSINSVESEDIADYYCQQNNNWPTTFGAGTKLELKGGGGSGGGGSGGGGSQVQLKQSGPGLVQPSQSLSITCTVSGFSLTNYGVHWVRQSPGKGLEWLGVIWSGGNTDYNTPFTSRLSINKDNSKSQVFFKMNSLQSNDTAIYYCARALTYYDYEFAYWGQGTLVTVSA

SEQ ID NO: 34 - protein, 243 aa, Artificial Sequence
  Synthetic Construct
DIKLQQSGAELARPGASVKMSCKTSGYTFTRYTMHWVKQRPGQGLEWIGYINPSRGYTNYNQKFKDKATLTTDKSSSTAYMQLSSLTSEDSAVYYCARYYDDHYCLDYWGQGTTLTVSSVEGGSGGSGGSGGSGGVDDIQLTQSPAIMSASPGEKVTMTCRASSSVSYMNWYQQKSGTSPKRWIYDTSKVASGVPYRFSGSGSGTSYSLTISSMEAEDAATYYCQQWSSNPLTFGAGTKLELK

SEQ ID NO: 35 - protein, 1009 aa, Artificial Sequence
  Synthetic Construct
EIQLVQSGAEVKKPGESLRISCKGSGFNIEDYYIHWVRQMPGKGLEWMGRIDPENDETKYGPIFQGHVTISADTSINTVYLQWSSLKASDTAMYYCAFRGGVYWGQGTTVTVSSGGGGSGGGGSGGGGSGGGGSDVVMTQSPDSLAVSLGERATINCKSSQSLLDSDGKTYLNWLQQKPGQPPKRLISLVSKLDSGVPDRFSGSGSGTDFTLTISSLQAEDVAVYYCWQGTHFPGTFGGGTKVEIKTTTPAPRPPTPAPTIASQPLSLRPEACRPAAGGAVHTRGLDFACDIYIWAPLAGTCGVLLLSLVITLYCKRGRKKLLYIFKQPFMRPVQTTQEEDGCSCRFPEEEEGGCELRVKFSRSADAPAYQQGQNQLYNELNLGRREEYDVLDKRRGRDPEMGGKPRRKNPQEGLYNELQKDKMAEAYSEIGMKGERRRGKGHDGLYQGLSTATKDTYDALHMQALPPRGSGATNFSLLKQAGDVEENPGPPRMETDTLLLWVLLLWVPGSTGDDILLTQSPVILSVSPGERVSFSCRASQSIGTNIHWYQQRTNGSPRLLIKYASESISGIPSRFSGSGSGTDFTLSINSVESEDIADYYCQQNNNWPTTFGAGTKLELKGGGGSGGGGSGGGGSQVQLKQSGPGLVQPSQSLSITCTVSGFSLTNYGVHWVRQSPGKGLEWLGVIWSGGNTDYNTPFTSRLSINKDNSKSQVFFKMNSLQSNDTAIYYCARALTYYDYEFAYWGQGTLVTVSAGGGGSDIKLQQSGAELARPGASVKMSCKTSGYTFTRYTMHWVKQRPGQGLEWIGYINPSRGYTNYNQKFKDKATLTTDKSSSTAYMQLSSLTSEDSAVYYCARYYDDHYCLDYWGQGTTLTVSSVEGGSGGSGGSGGSGGVDDIQLTQSPAIMSASPGEKVTMTCRASSSVSYMNWYQQKSGTSPKRWIYDTSKVASGVPYRFSGSGSGTSYSLTISSMEAEDAATYYCQQWSSNPLTFGAGTKLELKHHHHHH

SEQ ID NO: 36 - protein, 246 aa, Artificial Sequence
  Synthetic Construct
EIQLVQSGAEVKKPGESLRISCKGSGFNIEDYYIHWVRQMPGKGLEWMGRIDPENDETKYGPIFQGHVTISADTSINTVYLQWSSLKASDTAMYYCAFRGGVYWGQGTTVTVSSGGGGSGGGGSGGGGSGGGGSDVVMTQSPDSLAVSLGERATINCKSSQSLLDSDGKTYLNWLQQKPGQPPKRLISLVSKLDSGVPDRFSGSGSGTDFTLTISSLQAEDVAVYYCWQGTHFPGTFGGGTKVEIK

SEQ ID NO: 37 - protein, 69 aa, Artificial Sequence; identical to SEQ ID NO: 4
  Synthetic Construct

SEQ ID NO: 38 - protein, 42 aa, Artificial Sequence; identical to SEQ ID NO: 5
  Synthetic Construct

SEQ ID NO: 39 - protein, 112 aa, Artificial Sequence; identical to SEQ ID NO: 6
  Synthetic Construct

SEQ ID NO: 40 - protein, 22 aa, Artificial Sequence
  Synthetic Construct
GSGATNFSLLKQAGDVEENPGP

SEQ ID NO: 41 - protein, 21 aa, Artificial Sequence
  Synthetic Construct
METDTLLLWVLLLWVPGSTGD

SEQ ID NO: 42 - protein, 241 aa, Artificial Sequence; identical to SEQ ID NO: 33
  Synthetic Construct

SEQ ID NO: 43 - protein, 243 aa, Artificial Sequence; identical to SEQ ID NO: 34
  Synthetic Construct

SEQ ID NO: 44 - protein, 1018 aa, Artificial Sequence
  Synthetic Construct
EIQLVQSGAEVKKPGESLRISCKGSGFNIEDYYIHWVRQMPGKGLEWMGRIDPENDETKYGPIFQGHVTISADTSINTVYLQWSSLKASDTAMYYCAFRGGVYWGQGTTVTVSSGGGGSGGGGSGGGGSGGGGSDVVMTQSPDSLAVSLGERATINCKSSQSLLDSDGKTYLNWLQQKPGQPPKRLISLVSKLDSGVPDRFSGSGSGTDFTLTISSLQAEDVAVYYCWQGTHFPGTFGGGTKVEIKTTTPAPRPPTPAPTIASQPLSLRPEACRPAAGGAVHTRGLDFACDIYIWAPLAGTCGVLLLSLVITLYCKRGRKKLLYIFKQPFMRPVQTTQEEDGCSCRFPEEEEGGCELRVKFSRSADAPAYQQGQNQLYNELNLGRREEYDVLDKRRGRDPEMGGKPRRKNPQEGLYNELQKDKMAEAYSEIGMKGERRRGKGHDGLYQGLSTATKDTYDALHMQALPPRGSGATNFSLLKQAGDVEENPGPPRMETDTLLLWVLLLWVPGSTGDDIQLTQSPASLAVSLGQRATISCKASQSVDYDGDSYLNWYQQIPGQPPKLLIYDASNLVSGIPPRFSGSGSGTDFTLNIHPVEKVDAATYHCQQSTEDPWTFGGGTKLEIKGGGGSGGGGSGGGGSQVQLQQSGAELVRPGSSVKISCKASGYAFSSYWMNWVKQRPGQGLEWIGQIWPGDGDTNYNGKFKGKATLTADESSSTAYMQLSSLASEDSAVYFCARRETTTVGRYYYAMDYWGQGTTVTVSSGGGGSDIKLQQSGAELARPGASVKMSCKTSGYTFTRYTMHWVKQRPGQGLEWIGYINPSRGYTNYNQKFKDKATLTTDKSSSTAYMQLSSLTSEDSAVYYCARYYDDHYCLDYWGQGTTLTVSSVEGGSGGSGGSGGSGGVDDIQLTQSPAIMSASPGEKVTMTCRASSSVSYMNWYQQKSGTSPKRWIYDTSKVASGVPYRFSGSGSGTSYSLTISSMEAEDAATYYCQQWSSNPLTFGAGTKLELKHHHHHH

SEQ ID NO: 45 - protein, 246 aa, Artificial Sequence; identical to SEQ ID NO: 36
  Synthetic Construct

SEQ ID NO: 46 - protein, 69 aa, Artificial Sequence; identical to SEQ ID NO: 4
  Synthetic Construct

SEQ ID NO: 47 - protein, 42 aa, Artificial Sequence; identical to SEQ ID NO: 5
  Synthetic Construct

SEQ ID NO: 48 - protein, 112 aa, Artificial Sequence; identical to SEQ ID NO: 6
  Synthetic Construct

SEQ ID NO: 49 - protein, 22 aa, Artificial Sequence
  Synthetic Construct
GSGATNFSLLKQAGDVEENPGP

SEQ ID NO: 50 - protein, 21 aa, Artificial Sequence
  Synthetic Construct
METDTLLLWVLLLWVPGSTGD

SEQ ID NO: 51 - protein, 255 aa, Artificial Sequence
  Synthetic Construct
DIQLTQSPASLAVSLGQRATISCKASQSVDYDGDSYLNWYQQIPGQPPKLLIYDASNLVSGIPPRFSGSGSGTDFTLNIHPVEKVDAATYHCQQSTEDPWTFGGGTKLEIKGGGGSGGGGSGGGGSQVQLQQSGAELVRPGSSVKISCKASGYAFSSYWMNWVKQRPGQGLEWIGQIWPGDGDTNYNGKFKGKATLTADESSSTAYMQLSSLASEDSAVYFCARRETTTVGRYYYAMDYWGQGTTVTVSSGGGGS

SEQ ID NO: 52 - protein, 243 aa, Artificial Sequence; identical to SEQ ID NO: 34
  Synthetic Construct

SEQ ID NO: 53 - protein, 985 aa, Artificial Sequence
  Synthetic Construct
METDTLLLWVLLLWVPGSTGDDILLTQSPVILSVSPGERVSFSCRASQSIGTNIHWYQQRTNGSPRLLIKYASESISGIPSRFSGSGSGTDFTLSINSVESEDIADYYCQQNNNWPTTFGAGTKLELKGGGGSGGGGSGGGGSQVQLKQSGPGLVQPSQSLSITCTVSGFSLTNYGVHWVRQSPGKGLEWLGVIWSGGNTDYNTPFTSRLSINKDNSKSQVFFKMNSLQSNDTAIYYCARALTYYDYEFAYWGQGTLVTVSAGGGGSDIKLQQSGAELARPGASVKMSCKTSGYTFTRYTMHWVKQRPGQGLEWIGYINPSRGYTNYNQKFKDKATLTTDKSSSTAYMQLSSLTSEDSAVYYCARYYDDHYCLDYWGQGTTLTVSSVEGGSGGSGGSGGSGGVDDIQLTQSPAIMSASPGEKVTMTCRASSSVSYMNWYQQKSGTSPKRWIYDTSKVASGVPYRFSGSGSGTSYSLTISSMEAEDAATYYCQQWSSNPLTFGAGTKLELKHHHHHHEIQLVQSGAEVKKPGESLRISCKGSGFNIEDYYIHWVRQMPGKGLEWMGRIDPENDETKYGPIFQGHVTISADTSINTVYLQWSSLKASDTAMYYCAFRGGVYWGQGTTVTVSSGGGGSGGGGSGGGGSGGGGSDVVMTQSPDSLAVSLGERATINCKSSQSLLDSDGKTYLNWLQQKPGQPPKRLISLVSKLDSGVPDRFSGSGSGTDFTLTISSLQAEDVAVYYCWQGTHFPGTFGGGTKVEIKTTTPAPRPPTPAPTIASQPLSLRPEACRPAAGGAVHTRGLDFACDIYIWAPLAGTCGVLLLSLVITLYCKRGRKKLLYIFKQPFMRPVQTTQEEDGCSCRFPEEEEGGCELRVKFSRSADAPAYQQGQNQLYNELNLGRREEYDVLDKRRGRDPEMGGKPRRKNPQEGLYNELQKDKMAEAYSEIGMKGERRRGKGHDGLYQGLSTATKDTYDALHMQALPPR

SEQ ID NO: 54 - protein, 21 aa, Artificial Sequence
  Synthetic Construct
METDTLLLWVLLLWVPGSTGD

SEQ ID NO: 55 - protein, 241 aa, Artificial Sequence; identical to SEQ ID NO: 33
  Synthetic Construct

SEQ ID NO: 56 - protein, 243 aa, Artificial Sequence; identical to SEQ ID NO: 34
  Synthetic Construct

SEQ ID NO: 57 - protein, 246 aa, Artificial Sequence; identical to SEQ ID NO: 36
  Synthetic Construct

SEQ ID NO: 58 - protein, 69 aa, Artificial Sequence; identical to SEQ ID NO: 4
  Synthetic Construct

SEQ ID NO: 59 - protein, 42 aa, Artificial Sequence; identical to SEQ ID NO: 5
  Synthetic Construct

SEQ ID NO: 60 - protein, 112 aa, Artificial Sequence; identical to SEQ ID NO: 6
  Synthetic Construct

SEQ ID NO: 61 - protein, 994 aa, Artificial Sequence
  Synthetic Construct
METDTLLLWVLLLWVPGSTGDDIQLTQSPASLAVSLGQRATISCKASQSVDYDGDSYLNWYQQIPGQPPKLLIYDASNLVSGIPPRFSGSGSGTDFTLNIHPVEKVDAATYHCQQSTEDPWTFGGGTKLEIKGGGGSGGGGSGGGGSQVQLQQSGAELVRPGSSVKISCKASGYAFSSYWMNWVKQRPGQGLEWIGQIWPGDGDTNYNGKFKGKATLTADESSSTAYMQLSSLASEDSAVYFCARRETTTVGRYYYAMDYWGQGTTVTVSSGGGGSDIKLQQSGAELARPGASVKMSCKTSGYTFTRYTMHWVKQRPGQGLEWIGYINPSRGYTNYNQKFKDKATLTTDKSSSTAYMQLSSLTSEDSAVYYCARYYDDHYCLDYWGQGTTLTVSSVEGGSGGSGGSGGSGGVDDIQLTQSPAIMSASPGEKVTMTCRASSSVSYMNWYQQKSGTSPKRWIYDTSKVASGVPYRFSGSGSGTSYSLTISSMEAEDAATYYCQQWSSNPLTFGAGTKLELKHHHHHHEIQLVQSGAEVKKPGESLRISCKGSGFNIEDYYIHWVRQMPGKGLEWMGRIDPENDETKYGPIFQGHVTISADTSINTVYLQWSSLKASDTAMYYCAFRGGVYWGQGTTVTVSSGGGGSGGGGSGGGGSGGGGSDVVMTQSPDSLAVSLGERATINCKSSQSLLDSDGKTYLNWLQQKPGQPPKRLISLVSKLDSGVPDRFSGSGSGTDFTLTISSLQAEDVAVYYCWQGTHFPGTFGGGTKVEIKTTTPAPRPPTPAPTIASQPLSLRPEACRPAAGGAVHTRGLDFACDIYIWAPLAGTCGVLLLSLVITLYCKRGRKKLLYIFKQPFMRPVQTTQEEDGCSCRFPEEEEGGCELRVKFSRSADAPAYQQGQNQLYNELNLGRREEYDVLDKRRGRDPEMGGKPRRKNPQEGLYNELQKDKMAEAYSEIGMKGERRRGKGHDGLYQGLSTATKDTYDALHMQALPPR

SEQ ID NO: 62 - protein, 21 aa, Artificial Sequence
  Synthetic Construct
METDTLLLWVLLLWVPGSTGD

SEQ ID NO: 63 - protein, 250 aa, Artificial Sequence
  Synthetic Construct
DIQLTQSPASLAVSLGQRATISCKASQSVDYDGDSYLNWYQQIPGQPPKLLIYDASNLVSGIPPRFSGSGSGTDFTLNIHPVEKVDAATYHCQQSTEDPWTFGGGTKLEIKGGGGSGGGGSGGGGSQVQLQQSGAELVRPGSSVKISCKASGYAFSSYWMNWVKQRPGQGLEWIGQIWPGDGDTNYNGKFKGKATLTADESSSTAYMQLSSLASEDSAVYFCARRETTTVGRYYYAMDYWGQGTTVTVSS

SEQ ID NO: 64 - protein, 243 aa, Artificial Sequence; identical to SEQ ID NO: 34
  Synthetic Construct

SEQ ID NO: 65 - protein, 246 aa, Artificial Sequence; identical to SEQ ID NO: 36
  Synthetic Construct

SEQ ID NO: 66 - protein, 69 aa, Artificial Sequence; identical to SEQ ID NO: 4
  Synthetic Construct

SEQ ID NO: 67 - protein, 42 aa, Artificial Sequence; identical to SEQ ID NO: 5
  Synthetic Construct

SEQ ID NO: 68 - protein, 112 aa, Artificial Sequence; identical to SEQ ID NO: 6
  Synthetic Construct